European Patent Application EP 4 134 379 A1, published February 15, 2023. Title: ANTI-TRANSTHYRETIN ANTIBODIES. Applicant: Prothena Biosciences Limited. Application IB PCT/IB2016/050415, filed January 28, 2016. The sequence listing filed with the application follows.

SEQUENCE LISTING (118 sequences)

SEQ ID NO: 1 - protein, 124 aa, synthetic construct
  REGION 1..124: note = m9D5VH
EVKLVESGGGLVQPGGSLKLSCAASGFTFSSYTMSWVRQTPEKRLELVAEISNSGDTTYYPDTVKGRFTFSRDNAKNTLYLQMSSLKSEDTAMYYCARHYYYGGGYGGWFFDVWGTGTTVTVSS

SEQ ID NO: 2 - protein, 123 aa, synthetic construct
  REGION 1..123: note = 1SEQ_H
EVKLVESGGGLVQPGGSLKLSCAASGFTFSTYTMSWARQTPEKKLEWVAYISKGGGSTYYPDTVKGRFTISRDNAKNTLYLQMSSLKSEDTALYYCARGAMFGNDFKYPMDRWGQGTSVTVSS

SEQ ID NO: 3 - protein, 124 aa, synthetic construct
  REGION 1..124: note = BAC02114
EVQLVESGGGLVQPGGSLRLSCAASGFTFSSYEMNWVRQAPGKGLEWVSYITSSGSTIYYADSVKGRFTISRDNAKNSLYLQMNSLRAEDTAVYYCARGGQGSRYYYYYGMDVWGQGTTVTVSS

SEQ ID NO: 4 - protein, 120 aa, synthetic construct
  REGION 1..120: note = AAX82494
QVQLQESGGGLVKPGGSLKLSCAASGFTFSSYGMSWVRQTPDKRLEWVATISSGGSYTYYPDSVKGRFTISRDNAKNTLYLQMSSLKSEDTAMYYCARLYYGYRYYFDYWGQGTMVTVSS

SEQ ID NO: 5 - protein, 124 aa, synthetic construct
  REGION 1..124: note = Hu9D5VHv1
EVQLVESGGGLVQPGGSLRLSCAASGFTFSSYTMSWVRQAPGKGLELVAEISNSGDTTYYPDTVKGRFTFSRDNAKNSLYLQSNSLKAEDTAVYYCARHYYYGGGYGGWFFDVWGQGTTVTVSS

SEQ ID NO: 6 - protein, 124 aa, synthetic construct
  REGION 1..124: note = Hu9D5VHv2
EVQLVESGGGLVQPGGSLRLSCAASGFTFSSYTMSWVRQAPGKGLELVAEISNSGDTTYYPDTVKGRFTFSRDNAKNSLYLQSNLLRAEDTAVYYCARHYYYGGGYGGWFFDVWGQGTTVTVSS

SEQ ID NO: 7 - protein, 124 aa, synthetic construct
  REGION 1..124: note = Hu9D5VHv2b
EVQLVESGGGLVQPGGSLKLSCAASGFTFSSYTMSWVRQTPEKRLELVAEISNSGDTTYYPDTVKGRFTISRDNAKNTLYLQMSSLKSEDTAMYYCARHYYYGGGYGGWFFDVWGQGTLVTVSS

SEQ ID NO: 8 - protein, 124 aa, synthetic construct
  REGION 1..124: note = Hu9D5VHv3
EVQLVESGGGLVQPGGSLRLSCAASGFTFSSYTMSWVRQAPGKGLEWVSEISNSGDTTYYPDTVKGRFTFSRDNAKNSLYLQSNLLRAEDTAVYYCARHYYYGGGYGGWFFDVWGQGTTVTVSS

SEQ ID NO: 9 - protein, 124 aa, synthetic construct
  REGION 1..124: note = Hu9D5VHv3b
EVQLVESGGGLVQPGGSLKLSCAASGFTFSSYTMSWVRQTPGKRLELVAEISNSGDTTYYPDTVKGRFTISRDNAKNTLYLQMSSLKSEDTAMYYCARHYYYGGGYGGWFFDVWGQGTLVTVSS

SEQ ID NO: 10 - protein, 124 aa, synthetic construct
  REGION 1..124: note = Hu9D5VHv4
EVQLVESGGGLVQPGGSLRLSCAASGFTFSSYTMSWVRQAPGKGLEWVSEISNSGDTTYYPDTVKGRFTISRDNAKNSLYLQSNLLRAEDTAVYYCARHYYYGGGYGGWFFDVWGQGTTVTVSS

SEQ ID NO: 11 - protein, 124 aa, synthetic construct
  REGION 1..124: note = Hu9D5VHv4b
EVQLVESGGGLVQPGGSLKLSCAASGFTFSSYTMSWVRQAPGKRLELVAEISNSGDTTYYPDTVKGRFTISRDNAKNTLYLQMSSLKSEDTAMYYCARHYYYGGGYGGWFFDVWGQGTLVTVSS

SEQ ID NO: 12 - protein, 124 aa, synthetic construct
  REGION 1..124: note = Hu9D5VHv5
EVQLVESGGGLVQPGGSLRLSCAASGFTFSSYTMSWVRQTPEKRLELVAEISNSGDTTYYPDTVKGRFTISRDNAKNTLYLQMNLLRAEDTAVYYCARHYYYGGGYGGWFFDVWGQGTTVTVSS

SEQ ID NO: 13 - protein, 5 aa, synthetic construct
  REGION 1..5: note = 9D5 CDRH1 - Kabat
SYTMS

SEQ ID NO: 14 - protein, 17 aa, synthetic construct
  REGION 1..17: note = 9D5 CDRH2 - Kabat
EISNSGDTTYYPDTVKG

SEQ ID NO: 15 - protein, 15 aa, synthetic construct
  REGION 1..15: note = 9D5 CDRH3 - Kabat
HYYYGGGYGGWFFDV

SEQ ID NO: 16 - protein, 112 aa, synthetic construct
  REGION 1..112: note = m9D5VL
DIVMTQAAPSVPVTPGESVSISCRSSKSLLHSNGNTYLYWFLQRPGQSPQLLIYRVSNLASGVPDRFSGSGSGTAFTLRISRVEAEDVGVYYCMQHLEYPLTFGAGTKLELK

SEQ ID NO: 17 - protein, 112 aa, synthetic construct
  REGION 1..112: note = 1MJU_L
DIVMTQAAPSVPVTPGESVSISCRSSKSLLHSNGNTYLYWFLQRPGQSPQLLIYRMSNLASGVPDRFSGSGSGTAFTLRISRVEAEDVGVYYCLQHLEYPFTFGAGTKLELK

SEQ ID NO: 18 - protein, 112 aa, synthetic construct
  REGION 1..112: note = ABC66952
DIVMTQSPLSLPVTPGEPASISCRSNQSLLYSNGYNYLDWYLQKPGQSPQLLIYSGSNRASGVPDRFSGSGSGTDFTLKISRVEAEDVGVYYCMQALQSPYTFGQGTKLEIK

SEQ ID NO: 19 - protein, 112 aa, synthetic construct
  REGION 1..112: note = Hu9D5VLv1
DIVMTQSPLSLPVTPGEPASISCRSSKSLLHSNGNTYLYWFLQKPGQSPQLLIYRVSNLASGVPDRFSGSGSGTDFTLKISRVEAEDVGVYYCMQHLEYPLTFGQGTKLEIK

SEQ ID NO: 20 - protein, 112 aa, synthetic construct
  REGION 1..112: note = Hu9D5VLv2
DIVMTQSPLSLPVTPGEPASISCRSSKSLLHSNGNTYLYWYLQKPGQSPQLLIYRVSNLASGVPDRFSGSGSGTDFTLKISRVEAEDVGVYYCMQHLEYPLTFGQGTKLEIK

SEQ ID NO: 21 - protein, 112 aa, synthetic construct
  REGION 1..112: note = Hu9D5VLv3
DIVMTQSPLSLPVTPGEPASISCRSSKSLLHSNGNTYLYWYLQKPGQSPQLLIYRVSNLASGVPSRFSGSGSGTDFTLKISRVEAEDVGVYYCMQHLEYPLTFGQGTKLEIK

SEQ ID NO: 22 - protein, 112 aa, synthetic construct
  REGION 1..112: note = Hu9D5VLv4
DIVMTQSAPSLPVTPGEPVSISCRSSKSLLHSNGNTYLYWFLQRPGQSPQLLIYRVSNLASGVPSRFSGSGSGTAFTLRISRVEAEDVGVYYCMQHLEYPLTFGQGTKLEIK

SEQ ID NO: 23 - protein, 112 aa, synthetic construct
  REGION 1..112: note = Hu9D5VLv5
DIVMTQSAPSLPVTPGESVSISCRSSKSLLHSNGNTYLYWFLQRPGQSPQLLIYRVSNLASGVPSRFSGSGSGTAFTLRISRVEAEDVGVYYCMQHLEYPLTFGQGTKLEIK

SEQ ID NO: 24 - protein, 16 aa, synthetic construct
  REGION 1..16: note = 9D5 CDRL1 - Kabat
RSSKSLLHSNGNTYLY

SEQ ID NO: 25 - protein, 7 aa, synthetic construct
  REGION 1..7: note = 9D5 CDRL2 - Kabat
RVSNLAS

SEQ ID NO: 26 - protein, 9 aa, synthetic construct
  REGION 1..9: note = 9D5 CDRL3 - Kabat
MQHLEYPLT

SEQ ID NO: 27 - protein, 454 aa, synthetic construct
  REGION 1..454: note = Hu9D5 H1 heavy chain
EVQLVESGGGLVQPGGSLRLSCAASGFTFSSYTMSWVRQAPGKGLELVAEISNSGDTTYYPDTVKGRFTFSRDNAKNSLYLQSNSLKAEDTAVYYCARHYYYGGGYGGWFFDVWGQGTTVTVSSASTKGPSVFPLAPSSKSTSGGTAALGCLVKDYFPEPVTVSWNSGALTSGVHTFPAVLQSSGLYSLSSVVTVPSSSLGTQTYICNVNHKPSNTKVDKRVEPKSCDKTHTCPPCPAPELLGGPSVFLFPPKPKDTLMISRTPEVTCVVVDVSHEDPEVKFNWYVDGVEVHNAKTKPREEQYNSTYRVVSVLTVLHQDWLNGKEYKCKVSNKALPAPIEKTISKAKGQPREPQVYTLPPSREEMTKNQVSLTCLVKGFYPSDIAVEWESNGQPENNYKTTPPVLDSDGSFFLYSKLTVDKSRWQQGNVFSCSVMHEALHNHYTQKSLSLSPGK

SEQ ID NO: 28 - protein, 454 aa, synthetic construct
  REGION 1..454: note = Hu9D5 H2 heavy chain
EVQLVESGGGLVQPGGSLRLSCAASGFTFSSYTMSWVRQAPGKGLELVAEISNSGDTTYYPDTVKGRFTFSRDNAKNSLYLQSNLLRAEDTAVYYCARHYYYGGGYGGWFFDVWGQGTTVTVSSASTKGPSVFPLAPSSKSTSGGTAALGCLVKDYFPEPVTVSWNSGALTSGVHTFPAVLQSSGLYSLSSVVTVPSSSLGTQTYICNVNHKPSNTKVDKRVEPKSCDKTHTCPPCPAPELLGGPSVFLFPPKPKDTLMISRTPEVTCVVVDVSHEDPEVKFNWYVDGVEVHNAKTKPREEQYNSTYRVVSVLTVLHQDWLNGKEYKCKVSNKALPAPIEKTISKAKGQPREPQVYTLPPSREEMTKNQVSLTCLVKGFYPSDIAVEWESNGQPENNYKTTPPVLDSDGSFFLYSKLTVDKSRWQQGNVFSCSVMHEALHNHYTQKSLSLSPGK

SEQ ID NO: 29 - protein, 454 aa, synthetic construct
  REGION 1..454: note = Hu9D5 H2b heavy chain
EVQLVESGGGLVQPGGSLKLSCAASGFTFSSYTMSWVRQTPEKRLELVAEISNSGDTTYYPDTVKGRFTISRDNAKNTLYLQMSSLKSEDTAMYYCARHYYYGGGYGGWFFDVWGQGTLVTVSSASTKGPSVFPLAPSSKSTSGGTAALGCLVKDYFPEPVTVSWNSGALTSGVHTFPAVLQSSGLYSLSSVVTVPSSSLGTQTYICNVNHKPSNTKVDKRVEPKSCDKTHTCPPCPAPELLGGPSVFLFPPKPKDTLMISRTPEVTCVVVDVSHEDPEVKFNWYVDGVEVHNAKTKPREEQYNSTYRVVSVLTVLHQDWLNGKEYKCKVSNKALPAPIEKTISKAKGQPREPQVYTLPPSREEMTKNQVSLTCLVKGFYPSDIAVEWESNGQPENNYKTTPPVLDSDGSFFLYSKLTVDKSRWQQGNVFSCSVMHEALHNHYTQKSLSLSPGK

SEQ ID NO: 30 - protein, 454 aa, synthetic construct
  REGION 1..454: note = Hu9D5 H3 heavy chain
EVQLVESGGGLVQPGGSLRLSCAASGFTFSSYTMSWVRQAPGKGLEWVSEISNSGDTTYYPDTVKGRFTFSRDNAKNSLYLQSNLLRAEDTAVYYCARHYYYGGGYGGWFFDVWGQGTTVTVSSASTKGPSVFPLAPSSKSTSGGTAALGCLVKDYFPEPVTVSWNSGALTSGVHTFPAVLQSSGLYSLSSVVTVPSSSLGTQTYICNVNHKPSNTKVDKRVEPKSCDKTHTCPPCPAPELLGGPSVFLFPPKPKDTLMISRTPEVTCVVVDVSHEDPEVKFNWYVDGVEVHNAKTKPREEQYNSTYRVVSVLTVLHQDWLNGKEYKCKVSNKALPAPIEKTISKAKGQPREPQVYTLPPSREEMTKNQVSLTCLVKGFYPSDIAVEWESNGQPENNYKTTPPVLDSDGSFFLYSKLTVDKSRWQQGNVFSCSVMHEALHNHYTQKSLSLSPGK

SEQ ID NO: 31 - protein, 454 aa, synthetic construct
  REGION 1..454: note = Hu9D5 H3b heavy chain
EVQLVESGGGLVQPGGSLKLSCAASGFTFSSYTMSWVRQTPGKRLELVAEISNSGDTTYYPDTVKGRFTISRDNAKNTLYLQMSSLKSEDTAMYYCARHYYYGGGYGGWFFDVWGQGTLVTVSSASTKGPSVFPLAPSSKSTSGGTAALGCLVKDYFPEPVTVSWNSGALTSGVHTFPAVLQSSGLYSLSSVVTVPSSSLGTQTYICNVNHKPSNTKVDKRVEPKSCDKTHTCPPCPAPELLGGPSVFLFPPKPKDTLMISRTPEVTCVVVDVSHEDPEVKFNWYVDGVEVHNAKTKPREEQYNSTYRVVSVLTVLHQDWLNGKEYKCKVSNKALPAPIEKTISKAKGQPREPQVYTLPPSREEMTKNQVSLTCLVKGFYPSDIAVEWESNGQPENNYKTTPPVLDSDGSFFLYSKLTVDKSRWQQGNVFSCSVMHEALHNHYTQKSLSLSPGK

SEQ ID NO: 32 - protein, 454 aa, synthetic construct
  REGION 1..454: note = Hu9D5 H4 heavy chain
EVQLVESGGGLVQPGGSLRLSCAASGFTFSSYTMSWVRQAPGKGLEWVSEISNSGDTTYYPDTVKGRFTISRDNAKNSLYLQSNLLRAEDTAVYYCARHYYYGGGYGGWFFDVWGQGTTVTVSSASTKGPSVFPLAPSSKSTSGGTAALGCLVKDYFPEPVTVSWNSGALTSGVHTFPAVLQSSGLYSLSSVVTVPSSSLGTQTYICNVNHKPSNTKVDKRVEPKSCDKTHTCPPCPAPELLGGPSVFLFPPKPKDTLMISRTPEVTCVVVDVSHEDPEVKFNWYVDGVEVHNAKTKPREEQYNSTYRVVSVLTVLHQDWLNGKEYKCKVSNKALPAPIEKTISKAKGQPREPQVYTLPPSREEMTKNQVSLTCLVKGFYPSDIAVEWESNGQPENNYKTTPPVLDSDGSFFLYSKLTVDKSRWQQGNVFSCSVMHEALHNHYTQKSLSLSPGK

SEQ ID NO: 33 - protein, 454 aa, synthetic construct
  REGION 1..454: note = Hu9D5 H4b heavy chain
EVQLVESGGGLVQPGGSLKLSCAASGFTFSSYTMSWVRQAPGKRLELVAEISNSGDTTYYPDTVKGRFTISRDNAKNTLYLQMSSLKSEDTAMYYCARHYYYGGGYGGWFFDVWGQGTLVTVSSASTKGPSVFPLAPSSKSTSGGTAALGCLVKDYFPEPVTVSWNSGALTSGVHTFPAVLQSSGLYSLSSVVTVPSSSLGTQTYICNVNHKPSNTKVDKRVEPKSCDKTHTCPPCPAPELLGGPSVFLFPPKPKDTLMISRTPEVTCVVVDVSHEDPEVKFNWYVDGVEVHNAKTKPREEQYNSTYRVVSVLTVLHQDWLNGKEYKCKVSNKALPAPIEKTISKAKGQPREPQVYTLPPSREEMTKNQVSLTCLVKGFYPSDIAVEWESNGQPENNYKTTPPVLDSDGSFFLYSKLTVDKSRWQQGNVFSCSVMHEALHNHYTQKSLSLSPGK

SEQ ID NO: 34 - protein, 454 aa, synthetic construct
  REGION 1..454: note = Hu9D5 H5 heavy chain
EVQLVESGGGLVQPGGSLRLSCAASGFTFSSYTMSWVRQTPEKRLELVAEISNSGDTTYYPDTVKGRFTISRDNAKNTLYLQMNLLRAEDTAVYYCARHYYYGGGYGGWFFDVWGQGTTVTVSSASTKGPSVFPLAPSSKSTSGGTAALGCLVKDYFPEPVTVSWNSGALTSGVHTFPAVLQSSGLYSLSSVVTVPSSSLGTQTYICNVNHKPSNTKVDKRVEPKSCDKTHTCPPCPAPELLGGPSVFLFPPKPKDTLMISRTPEVTCVVVDVSHEDPEVKFNWYVDGVEVHNAKTKPREEQYNSTYRVVSVLTVLHQDWLNGKEYKCKVSNKALPAPIEKTISKAKGQPREPQVYTLPPSREEMTKNQVSLTCLVKGFYPSDIAVEWESNGQPENNYKTTPPVLDSDGSFFLYSKLTVDKSRWQQGNVFSCSVMHEALHNHYTQKSLSLSPGK

SEQ ID NO: 35 - protein, 219 aa, synthetic construct
  REGION 1..219: note = Hu9D5 L1 light chain
DIVMTQSPLSLPVTPGEPASISCRSSKSLLHSNGNTYLYWFLQKPGQSPQLLIYRVSNLASGVPDRFSGSGSGTDFTLKISRVEAEDVGVYYCMQHLEYPLTFGQGTKLEIKRTVAAPSVFIFPPSDEQLKSGTASVVCLLNNFYPREAKVQWKVDNALQSGNSQESVTEQDSKDSTYSLSSTLTLSKADYEKHKVYACEVTHQGLSSPVTKSFNRGEC

SEQ ID NO: 36 - protein, 219 aa, synthetic construct
  REGION 1..219: note = Hu9D5 L2 light chain
DIVMTQSPLSLPVTPGEPASISCRSSKSLLHSNGNTYLYWYLQKPGQSPQLLIYRVSNLASGVPDRFSGSGSGTDFTLKISRVEAEDVGVYYCMQHLEYPLTFGQGTKLEIKRTVAAPSVFIFPPSDEQLKSGTASVVCLLNNFYPREAKVQWKVDNALQSGNSQESVTEQDSKDSTYSLSSTLTLSKADYEKHKVYACEVTHQGLSSPVTKSFNRGEC

SEQ ID NO: 37 - protein, 219 aa, synthetic construct
  REGION 1..219: note = Hu9D5 L3 light chain
DIVMTQSPLSLPVTPGEPASISCRSSKSLLHSNGNTYLYWYLQKPGQSPQLLIYRVSNLASGVPSRFSGSGSGTDFTLKISRVEAEDVGVYYCMQHLEYPLTFGQGTKLEIKRTVAAPSVFIFPPSDEQLKSGTASVVCLLNNFYPREAKVQWKVDNALQSGNSQESVTEQDSKDSTYSLSSTLTLSKADYEKHKVYACEVTHQGLSSPVTKSFNRGEC

SEQ ID NO: 38 - protein, 219 aa, synthetic construct
  REGION 1..219: note = Hu9D5 L4 light chain
DIVMTQSAPSLPVTPGEPVSISCRSSKSLLHSNGNTYLYWFLQRPGQSPQLLIYRVSNLASGVPSRFSGSGSGTAFTLRISRVEAEDVGVYYCMQHLEYPLTFGQGTKLEIKRTVAAPSVFIFPPSDEQLKSGTASVVCLLNNFYPREAKVQWKVDNALQSGNSQESVTEQDSKDSTYSLSSTLTLSKADYEKHKVYACEVTHQGLSSPVTKSFNRGEC

SEQ ID NO: 39 - protein, 219 aa, synthetic construct
  REGION 1..219: note = Hu9D5 L5 light chain
DIVMTQSAPSLPVTPGESVSISCRSSKSLLHSNGNTYLYWFLQRPGQSPQLLIYRVSNLASGVPSRFSGSGSGTAFTLRISRVEAEDVGVYYCMQHLEYPLTFGQGTKLEIKRTVAAPSVFIFPPSDEQLKSGTASVVCLLNNFYPREAKVQWKVDNALQSGNSQESVTEQDSKDSTYSLSSTLTLSKADYEKHKVYACEVTHQGLSSPVTKSFNRGEC

SEQ ID NO: 40 - DNA, 429 bp, synthetic construct
  misc_feature 1..429: note = m9D5VH with signal peptide
  source 1..429: mol_type = other DNA
atggactttgggctcagcttgattttccttgtccttgttttaaaaggtgtcctgtgtgaagtgaagctggtggagtctgggggaggtttagtgcagcctggagggtccctgaaactctcctgtgcagcctctggattcactttcagtagctataccatgtcttgggttcgccagactccagaaaagaggctggagttggtcgcagaaattagtaatagtggtgataccacctactatccagacactgtaaagggccgattcaccttctccagagacaatgccaagaacaccctgtacctgcaaatgagcagtctgaagtctgaggacacggccatgtattactgtgcaagacattattactatggtggtggctacggggggtggttcttcgatgtctggggcacagggaccacggtcaccgtctcctcg

SEQ ID NO: 41 - protein, 143 aa, synthetic construct
  REGION 1..143: note = m9D5VH with signal peptide
MDFGLSLIFLVLVLKGVLCEVKLVESGGGLVQPGGSLKLSCAASGFTFSSYTMSWVRQTPEKRLELVAEISNSGDTTYYPDTVKGRFTFSRDNAKNTLYLQMSSLKSEDTAMYYCARHYYYGGGYGGWFFDVWGTGTTVTVSS

SEQ ID NO: 42 - DNA, 396 bp, synthetic construct
  misc_feature 1..396: note = m9D5VL with signal peptide
  source 1..396: mol_type = other DNA
atgaggtgcctagctgagttcctggggctgcttgtgctctggatccctggagccattggggatattgtgatgactcaggctgcaccctctgtacctgtcactcctggagagtcagtatccatctcctgcaggtctagtaagagtctcctgcatagtaatggcaacacttacttgtattggttcctgcagaggccaggccagtctcctcaactcctgatatatcgggtgtccaaccttgcctcaggagtcccagacaggttcagtggcagtgggtcaggaactgctttcacactgagaatcagtagagtggaggctgaggatgtgggtgtttattactgtatgcaacatttagaatatccgctcacgttcggtgctgggaccaagctggagctgaaa

SEQ ID NO: 43 - protein, 132 aa, synthetic construct
  REGION 1..132: note = m9D5VL with signal peptide
MRCLAEFLGLLVLWIPGAIGDIVMTQAAPSVPVTPGESVSISCRSSKSLLHSNGNTYLYWFLQRPGQSPQLLIYRVSNLASGVPDRFSGSGSGTAFTLRISRVEAEDVGVYYCMQHLEYPLTFGAGTKLELK

SEQ ID NO: 44 - DNA, 372 bp, synthetic construct
  misc_feature 1..372: note = Hu9D5VHv1
  source 1..372: mol_type = other DNA
gaggtgcagctggtggagtccggcggcggcctggtgcagcccggcggctccctgcgcctgtcctgcgccgcctccggcttcaccttctcctcctacaccatgtcctgggtgcgccaggcccccggcaagggcctggagctggtggccgagatctccaactccggcgacaccacctactaccccgacaccgtgaagggccgcttcaccttctcccgcgacaacgccaagaactccctgtacctgcagtccaactccctgaaggccgaggacaccgccgtgtactactgcgcccgccactactactacggcggcggctacggcggctggttcttcgacgtgtggggccagggcaccaccgtgaccgtgtcctca

SEQ ID NO: 45 - DNA, 372 bp, synthetic construct
  misc_feature 1..372: note = Hu9D5VHv2
  source 1..372: mol_type = other DNA
gaggtgcagctggtggagtccggcggcggcctggtgcagcccggcggctccctgcgcctgtcctgcgccgcctccggcttcaccttctcctcctacaccatgtcctgggtgcgccaggcccccggcaagggcctggagctggtggccgagatctccaactccggcgacaccacctactaccccgacaccgtgaagggccgcttcaccttctcccgcgacaacgccaagaactccctgtacctgcagtccaacctgctgcgcgccgaggacaccgccgtgtactactgcgcccgccactactactacggcggcggctacggcggctggttcttcgacgtgtggggccagggcaccaccgtgaccgtgtcctca

SEQ ID NO: 46 - DNA, 372 bp, synthetic construct
  misc_feature 1..372: note = Hu9D5VHv2b
  source 1..372: mol_type = other DNA
gaggtgcaactggtggagtctggcggcggcttggtgcaacctggcggctccctgaagctgtcctgtgccgcctccggcttcaccttcagcagctataccatgtcttgggtgcgccaaacccccgagaagaggctggagttggtggctgagattagtaatagcggcgataccacctactatcccgataccgtgaagggccgcttcaccatttccagagataatgctaagaataccctgtatctgcaaatgagtagcctgaagtctgaggataccgctatgtattattgtgctagacattattattatggcggcggctatggcggctggttcttcgatgtgtggggccaaggcaccctggtcaccgtgtcctca

SEQ ID NO: 47 - DNA, 372 bp, synthetic construct
  misc_feature 1..372: note = Hu9D5VHv3
  source 1..372: mol_type = other DNA
gaggtgcagctggtggagtccggcggcggcctggtgcagcccggcggctccctgcgcctgtcctgcgccgcctccggcttcaccttctcctcctacaccatgtcctgggtgcgccaggcccccggcaagggcctggagtgggtgtccgagatctccaactccggcgacaccacctactaccccgacaccgtgaagggccgcttcaccttctcccgcgacaacgccaagaactccctgtacctgcagtccaacctgctgcgcgccgaggacaccgccgtgtactactgcgcccgccactactactacggcggcggctacggcggctggttcttcgacgtgtggggccagggcaccaccgtgaccgtgtcctca

SEQ ID NO: 48 - DNA, 372 bp, synthetic construct
  misc_feature 1..372: note = Hu9D5VHv3b
  source 1..372: mol_type = other DNA
gaggtgcaactggtggagtctggcggcggcttggtgcaacctggcggctccctgaagctgtcctgtgccgcctccggcttcaccttcagcagctataccatgtcttgggtgcgccaaacccccgggaagaggctggagttggtggctgagattagtaatagcggcgataccacctactatcccgataccgtgaagggccgcttcaccatttccagagataatgctaagaataccctgtatctgcaaatgagtagcctgaagtctgaggataccgctatgtattattgtgctagacattattattatggcggcggctatggcggctggttcttcgatgtgtggggccaaggcaccctggtcaccgtgtcctca

SEQ ID NO: 49 - DNA, 372 bp, synthetic construct
  misc_feature 1..372: note = Hu9D5VHv4
  source 1..372: mol_type = other DNA
gaggtgcagctggtggagtccggcggcggcctggtgcagcccggcggctccctgcgcctgtcctgcgccgcctccggcttcaccttctcctcctacaccatgtcctgggtgcgccaggcccccggcaagggcctggagtgggtgtccgagatctccaactccggcgacaccacctactaccccgacaccgtgaagggccgcttcaccatctcccgcgacaacgccaagaactccctgtacctgcagtccaacctgctgcgcgccgaggacaccgccgtgtactactgcgcccgccactactactacggcggcggctacggcggctggttcttcgacgtgtggggccagggcaccaccgtgaccgtgtcctca

SEQ ID NO: 50 - DNA, 372 bp, synthetic construct
  misc_feature 1..372: note = Hu9D5VHv4b
  source 1..372: mol_type = other DNA
gaggtgcaactggtggagtctggcggcggcttggtgcaacctggcggctccctgaagctgtcctgtgccgcctccggcttcaccttcagcagctataccatgtcttgggtgcgccaagcccccgggaagaggctggagttggtggctgagattagtaatagcggcgataccacctactatcccgataccgtgaagggccgcttcaccatttccagagataatgctaagaataccctgtatctgcaaatgagtagcctgaagtctgaggataccgctatgtattattgtgctagacattattattatggcggcggctatggcggctggttcttcgatgtgtggggccaaggcaccctggtcaccgtgtcctca

SEQ ID NO: 51 - DNA, 372 bp, synthetic construct
  misc_feature 1..372: note = Hu9D5VHv5
  source 1..372: mol_type = other DNA
gaggtgcagctggtggagtccggcggcggcctggtgcagcccggcggctccctgcgcctgtcctgcgccgcctccggcttcaccttctcctcctacaccatgtcctgggtgcgccagacccccgagaagcgcctggagctggtggccgagatctccaactccggcgacaccacctactaccccgacaccgtgaagggccgcttcaccatctcccgcgacaacgccaagaacaccctgtacctgcagatgaacctgctgcgcgccgaggacaccgccgtgtactactgcgcccgccactactactacggcggcggctacggcggctggttcttcgacgtgtggggccaaggcaccaccgtgaccgtgtcctca

SEQ ID NO: 52 - DNA, 336 bp, synthetic construct
  misc_feature 1..336: note = Hu9D5VLv1
  source 1..336: mol_type = other DNA
gacatcgtgatgacccagtcccccctgtccctgcccgtgacccccggcgagcccgcctccatctcctgccgctcctccaagtccctgctgcactccaacggcaacacctacctgtactggttcctgcagaagcccggccagtccccccagctgctgatctaccgcgtgtccaacctggcctccggcgtgcccgaccgcttctccggctccggctccggcaccgacttcaccctgaagatctcccgcgtggaggccgaggacgtgggcgtgtactactgcatgcagcacctggagtaccccctgaccttcggccagggcaccaagctggagatcaaa

SEQ ID NO: 53 - DNA, 336 bp, synthetic construct
  misc_feature 1..336: note = Hu9D5VLv2
  source 1..336: mol_type = other DNA
gacatcgtgatgacccagtcccccctgtccctgcccgtgacccccggcgagcccgcctccatctcctgccgctcctccaagtccctgctgcactccaacggcaacacctacctgtactggtacctgcagaagcccggccagtccccccagctgctgatctaccgcgtgtccaacctggcctccggcgtgcccgaccgcttctccggctccggctccggcaccgacttcaccctgaagatctcccgcgtggaggccgaggacgtgggcgtgtactactgcatgcagcacctggagtaccccctgaccttcggccagggcaccaagctggagatcaaa

SEQ ID NO: 54 - DNA, 336 bp, synthetic construct
  misc_feature 1..336: note = Hu9D5VLv3
  source 1..336: mol_type = other DNA
gacatcgtgatgacccagtcccccctgtccctgcccgtgacccccggcgagcccgcctccatctcctgccgctcctccaagtccctgctgcactccaacggcaacacctacctgtactggtacctgcagaagcccggccagtccccccagctgctgatctaccgcgtgtccaacctggcctccggcgtgccctcccgcttctccggctccggctccggcaccgacttcaccctgaagatctcccgcgtggaggccgaggacgtgggcgtgtactactgcatgcagcacctggagtaccccctgaccttcggccagggcaccaagctggagatcaaa

SEQ ID NO: 55 - DNA, 336 bp, synthetic construct
  misc_feature 1..336: note = Hu9D5VLv4
  source 1..336: mol_type = other DNA
gacatcgtgatgacccagtccgccccctccctgcccgtgacccccggcgagcccgtgtccatctcctgccgctcctccaagtccctgctgcactccaacggcaacacctacctgtactggttcctgcagcgccccggccagtccccccagctgctgatctaccgcgtgtccaacctggcctccggcgtgccctcccgcttctccggctccggctccggcaccgccttcaccctgcgcatctcccgcgtggaggccgaggacgtgggcgtgtactactgcatgcagcacctggagtaccccctgaccttcggccaaggcaccaagctggagatcaaa

SEQ ID NO: 56 - DNA, 336 bp, synthetic construct
  misc_feature 1..336: note = Hu9D5VLv5
  source 1..336: mol_type = other DNA
gacatcgtgatgacccagtccgccccctccctgcccgtgacccccggcgagtccgtgtccatctcctgccgctcctccaagtccctgctgcactccaacggcaacacctacctgtactggttcctgcagcgccccggccagtccccccagctgctgatctaccgcgtgtccaacctggcctccggcgtgccctcccgcttctccggctccggctccggcaccgccttcaccctgcgcatctcccgcgtggaggccgaggacgtgggcgtgtactactgcatgcagcacctggagtaccccctgaccttcggccaaggcaccaagctggagatcaaa

SEQ ID NO: 57 - protein, 19 aa, synthetic construct
  REGION 1..19: note = 9D5VH Signal Peptide
MDFGLSLIFLVLVLKGVLC

SEQ ID NO: 58 - DNA, 57 bp, synthetic construct
  misc_feature 1..57: note = 9D5VH Signal Peptide
  source 1..57: mol_type = other DNA
atggactttgggctcagcttgattttccttgtccttgttttaaaaggtgtcctgtgt

SEQ ID NO: 59 - protein, 20 aa, synthetic construct
  REGION 1..20: note = 9D5VL Signal Peptide
MRCLAEFLGLLVLWIPGAIG

SEQ ID NO: 60 - DNA, 60 bp, synthetic construct
  misc_feature 1..60: note = 9D5VL Signal Peptide
  source 1..60: mol_type = other DNA
atgaggtgcctagctgagttcctggggctgcttgtgctctggatccctggagccattggg

SEQ ID NO: 61 - protein, 124 aa, synthetic construct
  REGION 1..124: note = m14G8VH
EVKLVESGGGLVQPGGSLKLSCAASGFTFSSYTMSWVRQTPEKRLELVAEINNSGDTTYYPDTVKGRFTISRDNAKNTLYLQMSSLKSEDTAMYYCARHYYYGGGYGGWFFDVWGTGTTVTVSS

SEQ ID NO: 62 - protein, 118 aa, synthetic construct
  REGION 1..118: note = 1MQK_H
EVKLQESGGDLVQPGGSLKLSCAASGFTFSSYTMSWVRQTPEKRLEWVASINNGGGRTYYPDTVKGRFTISRDNAKNTLYLQMSSLKSEDTAMYYCVRHEYYYAMDYWGQGTTVTVSS

SEQ ID NO: 63 - protein, 124 aa, synthetic construct
  REGION 1..124: note = AAD30410
QVQLVQSGGGLVQPGGSRKLSCAASGFTFSSYAMSWVRQTPEKRLEWVAAISTDGSFIYYADTVKGRFTISGDNSKNTLYLQMNSLRAEDTAVYYCAKDRGIDATAQVGRFDPWGQGTLVTVSS

SEQ ID NO: 64 - protein, 124 aa, synthetic construct
  REGION 1..124: note = Hu14G8VHv1
EVKLVESGGGLVQPGGSLKLSCAASGFTFSSYTMSWVRQTPEKRLELVAEINNSGDTTYYPDTVKGRFTISRDNAKNTLYLQMSSLKSEDTAMYYCARHYYYGGGYGGWFFDVWGTGTLVTVSS

SEQ ID NO: 65 - protein, 124 aa, synthetic construct
  REGION 1..124: note = Hu14G8VHv2
EVQLVESGGGLVQPGGSLKLSCAASGFTFSSYTMSWVRQTPEKRLELVAEINNSGDTTYYPDTVKGRFTISRDNAKNTLYLQMSSLKSEDTAMYYCARHYYYGGGYGGWFFDVWGQGTLVTVSS

SEQ ID NO: 66 - protein, 124 aa, synthetic construct
  REGION 1..124: note = Hu14G8VHv3
EVQLVESGGGLVQPGGSLKLSCAASGFTFSSYTMSWVRQTPEKRLELVAEINNSGDTTYYPDTVKGRFTISRDNAKNTLYLQMNSLRAEDTAVYYCARHYYYGGGYGGWFFDVWGQGTLVTVSS

SEQ ID NO: 67 - protein, 5 aa, synthetic construct
  REGION 1..5: note = 14G8 CDRH1 - Kabat
SYTMS

SEQ ID NO: 68 - protein, 17 aa, synthetic construct
  REGION 1..17: note = 14G8 CDRH2 - Kabat
EINNSGDTTYYPDTVKG

SEQ ID NO: 69 - protein, 15 aa, synthetic construct
  REGION 1..15: note = 14G8 CDRH3 - Kabat
HYYYGGGYGGWFFDV

SEQ ID NO: 70 - protein, 113 aa, synthetic construct
  REGION 1..113: note = m14G8VL
DIVMTQAAPSVPVTPGESVSISCRSNKSLLHSNGNTYLYWFLQRPGQSPQLLIYRVSNLASGVPDRFSGSGSGTAFTLRISRVEAEDVGVYYCMQHLEYPLTFGAGTKLELKR

SEQ ID NO: 71 - protein, 113 aa, synthetic construct
  REGION 1..113: note = MJU_L
DIVMTQAAPSVPVTPGESVSISCRSSKSLLHSNGNTYLYWFLQRPGQSPQLLIYRMSNLASGVPDRFSGSGSGTAFTLRISRVEAEDVGVYYCLQHLEYPFTFGAGTKLELKR

SEQ ID NO: 72 - protein, 113 aa, synthetic construct
  REGION 1..113: note = ABA71374
DIVMTQTPLSLPVTPGESASISCRSSQSLRHYSGYTYIDWYLQKPGQSPQVLIYLGSNRASGVPDRFSGSGSGTDFTLKISRVEAEDVGVYYCMQALQTVCSFGQGTKLEIKR

SEQ ID NO: 73 - protein, 113 aa, synthetic construct
  REGION 1..113: note = ABC66952
DIVMTQSPLSLPVTPGEPASISCRSNQSLLYSNGYNYLDWYLQKPGQSPQLLIYSGSNRASGVPDRFSGSGSGTDFTLKISRVEAEDVGVYYCMQALQSPYTFGQGTKLEIKR

SEQ ID NO: 74 - protein, 113 aa, synthetic construct
  REGION 1..113: note = Hu14G8VLv1
DIVMTQSAPSLPVTPGESVSISCRSNKSLLHSNGNTYLYWFLQKPGQSPQLLIYRVSNLASGVPDRFSGSGSGTAFTLKISRVEAEDVGVYYCMQHLEYPLTFGQGTKLEIKR

SEQ ID NO: 75 - protein, 113 aa, synthetic construct
  REGION 1..113: note = Hu14G8VLv2
DIVMTQSPLSLPVTPGEPASISCRSNKSLLHSNGNTYLYWFLQKPGQSPQLLIYRVSNLASGVPDRFSGSGSGTDFTLKISRVEAEDVGVYYCMQHLEYPLTFGQGTKLEIKR

SEQ ID NO: 76 - protein, 113 aa, synthetic construct
  REGION 1..113: note = Hu14G8VLv3
DIVMTQSPLSLPVTPGEPASISCRSSKSLLHSNGNTYLYWFLQKPGQSPQLLIYRVSNLASGVPSRFSGSGSGTDFTLKISRVEAEDVGVYYCMQHLEYPLTFGQGTKLEIKR

SEQ ID NO: 77 - protein, 16 aa, synthetic construct
  REGION 1..16: note = 14G8 CDRL1 (mouse, HuVLv1, HuVLv2) - Kabat
RSNKSLLHSNGNTYLY

SEQ ID NO: 78 - protein, 7 aa, synthetic construct
  REGION 1..7: note = 14G8 CDRL2 - Kabat
RVSNLAS

SEQ ID NO: 79 - protein, 9 aa, synthetic construct
  REGION 1..9: note = 14G8 CDRL3 - Kabat
MQHLEYPLT

SEQ ID NO: 80 - protein, 16 aa, synthetic construct
  REGION 1..16: note = 14G8 CDRL1 (HuVLv3) - Kabat
RSSKSLLHSNGNTYLY

SEQ ID NO: 81 - protein, 454 aa, synthetic construct
  REGION 1..454: note = Hu14G8 H1 heavy chain
EVKLVESGGGLVQPGGSLKLSCAASGFTFSSYTMSWVRQTPEKRLELVAEINNSGDTTYYPDTVKGRFTISRDNAKNTLYLQMSSLKSEDTAMYYCARHYYYGGGYGGWFFDVWGTGTLVTVSSASTKGPSVFPLAPSSKSTSGGTAALGCLVKDYFPEPVTVSWNSGALTSGVHTFPAVLQSSGLYSLSSVVTVPSSSLGTQTYICNVNHKPSNTKVDKRVEPKSCDKTHTCPPCPAPELLGGPSVFLFPPKPKDTLMISRTPEVTCVVVDVSHEDPEVKFNWYVDGVEVHNAKTKPREEQYNSTYRVVSVLTVLHQDWLNGKEYKCKVSNKALPAPIEKTISKAKGQPREPQVYTLPPSREEMTKNQVSLTCLVKGFYPSDIAVEWESNGQPENNYKTTPPVLDSDGSFFLYSKLTVDKSRWQQGNVFSCSVMHEALHNHYTQKSLSLSPGK

SEQ ID NO: 82 - protein, 454 aa, synthetic construct
  REGION 1..454: note = Hu14G8 H2 heavy chain
EVQLVESGGGLVQPGGSLKLSCAASGFTFSSYTMSWVRQTPEKRLELVAEINNSGDTTYYPDTVKGRFTISRDNAKNTLYLQMSSLKSEDTAMYYCARHYYYGGGYGGWFFDVWGQGTLVTVSSASTKGPSVFPLAPSSKSTSGGTAALGCLVKDYFPEPVTVSWNSGALTSGVHTFPAVLQSSGLYSLSSVVTVPSSSLGTQTYICNVNHKPSNTKVDKRVEPKSCDKTHTCPPCPAPELLGGPSVFLFPPKPKDTLMISRTPEVTCVVVDVSHEDPEVKFNWYVDGVEVHNAKTKPREEQYNSTYRVVSVLTVLHQDWLNGKEYKCKVSNKALPAPIEKTISKAKGQPREPQVYTLPPSREEMTKNQVSLTCLVKGFYPSDIAVEWESNGQPENNYKTTPPVLDSDGSFFLYSKLTVDKSRWQQGNVFSCSVMHEALHNHYTQKSLSLSPGK

SEQ ID NO: 83 - protein, 454 aa, synthetic construct
  REGION 1..454: note = Hu14G8 H3 heavy chain
EVQLVESGGGLVQPGGSLKLSCAASGFTFSSYTMSWVRQTPEKRLELVAEINNSGDTTYYPDTVKGRFTISRDNAKNTLYLQMNSLRAEDTAVYYCARHYYYGGGYGGWFFDVWGQGTLVTVSSASTKGPSVFPLAPSSKSTSGGTAALGCLVKDYFPEPVTVSWNSGALTSGVHTFPAVLQSSGLYSLSSVVTVPSSSLGTQTYICNVNHKPSNTKVDKRVEPKSCDKTHTCPPCPAPELLGGPSVFLFPPKPKDTLMISRTPEVTCVVVDVSHEDPEVKFNWYVDGVEVHNAKTKPREEQYNSTYRVVSVLTVLHQDWLNGKEYKCKVSNKALPAPIEKTISKAKGQPREPQVYTLPPSREEMTKNQVSLTCLVKGFYPSDIAVEWESNGQPENNYKTTPPVLDSDGSFFLYSKLTVDKSRWQQGNVFSCSVMHEALHNHYTQKSLSLSPGK

SEQ ID NO: 84 - protein, 219 aa, synthetic construct
  REGION 1..219: note = Hu14G8 L1 light chain
DIVMTQSAPSLPVTPGESVSISCRSNKSLLHSNGNTYLYWFLQKPGQSPQLLIYRVSNLASGVPDRFSGSGSGTAFTLKISRVEAEDVGVYYCMQHLEYPLTFGQGTKLEIKRTVAAPSVFIFPPSDEQLKSGTASVVCLLNNFYPREAKVQWKVDNALQSGNSQESVTEQDSKDSTYSLSSTLTLSKADYEKHKVYACEVTHQGLSSPVTKSFNRGEC

SEQ ID NO: 85 - protein, 219 aa, synthetic construct
  REGION 1..219: note = Hu14G8 L2 light chain
DIVMTQSPLSLPVTPGEPASISCRSNKSLLHSNGNTYLYWFLQKPGQSPQLLIYRVSNLASGVPDRFSGSGSGTDFTLKISRVEAEDVGVYYCMQHLEYPLTFGQGTKLEIKRTVAAPSVFIFPPSDEQLKSGTASVVCLLNNFYPREAKVQWKVDNALQSGNSQESVTEQDSKDSTYSLSSTLTLSKADYEKHKVYACEVTHQGLSSPVTKSFNRGEC

SEQ ID NO: 86 - protein, 219 aa, synthetic construct
  REGION 1..219: note = Hu14G8 L3 light chain
DIVMTQSPLSLPVTPGEPASISCRSSKSLLHSNGNTYLYWFLQKPGQSPQLLIYRVSNLASGVPSRFSGSGSGTDFTLKISRVEAEDVGVYYCMQHLEYPLTFGQGTKLEIKRTVAAPSVFIFPPSDEQLKSGTASVVCLLNNFYPREAKVQWKVDNALQSGNSQESVTEQDSKDSTYSLSSTLTLSKADYEKHKVYACEVTHQGLSSPVTKSFNRGEC

SEQ ID NO: 87 - DNA, 429 bp, synthetic construct
  misc_feature 1..429: note = m14G8VH with signal peptide
  source 1..429: mol_type = other DNA
atgaatttcgggctcagcttgattttccttgtccttgttttaaaaggtgtcctgtgtgaagtgaagctggtggagtctgggggaggtttagtgcagcctggagggtccctgaaactctcctgtgcagcctccggattcactttcagtagctataccatgtcttgggttcgccagactccagaaaagaggctggagttggtcgcagaaattaataatagtggtgataccacctactatccagacactgtaaagggccgattcaccatctccagagacaatgccaagaacaccctgtacctgcaaatgagcagtctgaagtctgaggacacggccatgtattactgtgcaagacattattactatggtggtggctacggggggtggttcttcgatgtctggggcacagggaccacggtcaccgtctcctca

SEQ ID NO: 88 - protein, 143 aa, synthetic construct
  REGION 1..143: note = m14G8VH with signal peptide
MNFGLSLIFLVLVLKGVLCEVKLVESGGGLVQPGGSLKLSCAASGFTFSSYTMSWVRQTPEKRLELVAEINNSGDTTYYPDTVKGRFTISRDNAKNTLYLQMSSLKSEDTAMYYCARHYYYGGGYGGWFFDVWGTGTTVTVSS

SEQ ID NO: 89 - DNA, 399 bp, synthetic construct
  misc_feature 1..399: note = m14G8VL with signal peptide
  source 1..399: mol_type = other DNA
atgaggtgcctagctgagttcctggggctgcttgtgctctggatccctggagccattggggatattgtgatgactcaggctgcaccctctgtacctgtcactcctggagagtcagtatccatctcctgcaggtctaataagagtctcctgcatagtaatggcaacacttacttgtattggttcctgcagaggccaggccagtctcctcaactcctgatatatcgggtgtccaaccttgcctcaggagtcccagacaggttcagtggcagtgggtcaggaactgctttcacactgagaatcagtagagtggaggctgaggatgtgggtgtttattactgtatgcaacatttagaatatccgctcacgttcggtgctgggaccaagctggagctgaaacgt

SEQ ID NO: 90 - protein, 133 aa, synthetic construct
  REGION 1..133: note = m14G8VL with signal peptide
MRCLAEFLGLLVLWIPGAIGDIVMTQAAPSVPVTPGESVSISCRSNKSLLHSNGNTYLYWFLQRPGQSPQLLIYRVSNLASGVPDRFSGSGSGTAFTLRISRVEAEDVGVYYCMQHLEYPLTFGAGTKLELKR

SEQ ID NO: 91 - DNA, 372 bp, synthetic construct
  misc_feature 1..372: note = Hu14G8VHv1
  source 1..372: mol_type = other DNA
gaggtgaagctggtggagtctggcggcggcttggtgcaacctggcggctccctgaagctgtcctgtgccgcctccggcttcaccttcagcagctataccatgtcttgggtgcgccaaacccccgagaagaggctggagttggtggctgagattaataatagcggcgataccacctactatcccgataccgtgaagggccgcttcaccatttccagagataatgctaagaataccctgtatctgcaaatgagtagcctgaagtctgaggataccgctatgtattattgtgctagacattattattatggcggcggctatggcggctggttcttcgatgtgtggggcaccggcaccctggtcaccgtgtcctca

SEQ ID NO: 92 - DNA, 372 bp, synthetic construct
  misc_feature 1..372: note = Hu14G8VHv2
  source 1..372: mol_type = other DNA
gaggtgcaactggtggagtctggcggcggcttggtgcaacctggcggctccctgaagctgtcctgtgccgcctccggcttcaccttcagcagctataccatgtcttgggtgcgccaaacccccgagaagaggctggagttggtggctgagattaataatagcggcgataccacctactatcccgataccgtgaagggccgcttcaccatttccagagataatgctaagaataccctgtatctgcaaatgagtagcctgaagtctgaggataccgctatgtattattgtgctagacattattattatggcggcggctatggcggctggttcttcgatgtgtggggccaaggcaccctggtcaccgtgtcctca

SEQ ID NO: 93 - DNA, 372 bp, synthetic construct
  misc_feature 1..372: note = Hu14G8VHv3
  source 1..372: mol_type = other DNA
gaggtgcaactggtggagtctggcggcggcttggtgcaacctggcggctccctgaagctgtcctgtgccgcctccggcttcaccttcagcagctataccatgtcttgggtgcgccaaacccccgagaagaggctggagttggtggctgagattaataatagcggcgataccacctactatcccgataccgtgaagggccgcttcaccatttccagagataatgctaagaataccctgtatctgcaaatgaatagcctgagggctgaggataccgctgtgtattattgtgctagacattattattatggcggcggctatggcggctggttcttcgatgtgtggggccaaggcaccctggtcaccgtgtcctca

SEQ ID NO: 94 - DNA, 339 bp, synthetic construct
  misc_feature 1..339: note = Hu14G8VLv1
  source 1..339: mol_type = other DNA
gatatcgtgatgacccagtctgccccctccctgcctgtgacccctggcgagtccgtgtccatctcctgccggtccaacaagagcctgctgcacagcaacggcaacacctacctgtactggttcctgcaaaagcccggccaatcccctcaactgctgatctaccgggtgtccaacctggcctccggcgtgcccgataggttctccggaagcggctccggcaccgccttcaccctgaagattagtagagtcgaggccgaggatgtgggcgtgtactactgtatgcaacacttggagtaccccctgacgttcggccaaggcaccaagctggagatcaagcgt

SEQ ID NO: 95 - DNA, 339 bp, synthetic construct
  misc_feature 1..339: note = Hu14G8VLv2
  source 1..339: mol_type = other DNA
gatatcgtgatgacccagtctcccctgtccctgcctgtgacccctggcgagcccgcctccatctcctgccggtccaacaagagcctgctgcacagcaacggcaacacctacctgtactggttcctgcaaaagcccggccaatcccctcaactgctgatctaccgggtgtccaacctggcctccggcgtgcccgataggttctccggaagcggctccggcaccgatttcaccctgaagattagtagagtcgaggccgaggatgtgggcgtgtactactgtatgcaacacttggagtaccccctgacgttcggccaaggcaccaagctggagatcaagcgt

SEQ ID NO: 96 - DNA, 339 bp, synthetic construct
  misc_feature 1..339: note = Hu14G8VLv3
  source 1..339: mol_type = other DNA
gatatcgtgatgacccagtctcccctgtccctgcctgtgacccctggcgagcccgcctccatctcctgccggtccagcaagagcctgctgcacagcaacggcaacacctacctgtactggttcctgcaaaagcccggccaatcccctcaactgctgatctaccgggtgtccaacctggcctccggcgtgcccagtaggttctccggaagcggctccggcaccgatttcaccctgaagattagtagagtcgaggccgaggatgtgggcgtgtactactgtatgcaacacttggagtaccccctgacgttcggccaaggcaccaagctggagatcaagcgt

SEQ ID NO: 97 - protein, 19 aa, synthetic construct
  REGION 1..19: note = 14G8VH Signal Peptide
MNFGLSLIFLVLVLKGVLC

SEQ ID NO: 98 - DNA, 57 bp, synthetic construct
  misc_feature 1..57: note = 14G8VH Signal Peptide
  source 1..57: mol_type = other DNA
atgaatttcggcctgagcttgattttcctggtgctggtgttgaagggcgtgctgtgt

SEQ ID NO: 99 - protein, 20 aa, synthetic construct
  REGION 1..20: note = 14G8VL Signal Peptide
MRCLAEFLGLLVLWIPGAIG

SEQ ID NO: 100 - DNA, 60 bp, synthetic construct
  misc_feature 1..60: note = 14G8VL Signal Peptide
  source 1..60: mol_type = other DNA
atgaggtgcctggccgagttcctgggcctgctggtgctgtggatccctggcgccatcggc

SEQ ID NO: 101 - protein, 330 aa, synthetic construct
  REGION 1..330: note = Human IgG1 heavy chain constant region
ASTKGPSVFPLAPSSKSTSGGTAALGCLVKDYFPEPVTVSWNSGALTSGVHTFPAVLQSSGLYSLSSVVTVPSSSLGTQTYICNVNHKPSNTKVDKRVEPKSCDKTHTCPPCPAPELLGGPSVFLFPPKPKDTLMISRTPEVTCVVVDVSHEDPEVKFNWYVDGVEVHNVKTKPREEQYNSTYRVVSVLTVLHQDWLNGKEYKCKVSNKALPAPIEKTISKAKGQPREPQVYTLPPSREEMTKNQVSLTCLVKGFYPSDIAVEWESNGQPENNYKTTPPVLDSDGSFFLYSKLTVDKSRWQQGNVFSCSVMHEALHNHYTQKSLSLSPGK

SEQ ID NO: 102 - protein, 330 aa, synthetic construct
  REGION 1..330: note = Human IgG1 heavy chain constant region of IgG1G1m3 allotype
ASTKGPSVFPLAPSSKSTSGGTAALGCLVKDYFPEPVTVSWNSGALTSGVHTFPAVLQSSGLYSLSSVVTVPSSSLGTQTYICNVNHKPSNTKVDKRVEPKSCDKTHTCPPCPAPEAAGGPSVFLFPPKPKDTLMISRTPEVTCVVVDVSHEDPEVKFNWYVDGVEVHNAKTKPREEQYNSTYRVVSVLTVLHQDWLNGKEYKCKVSNKALPAPIEKTISKAKGQPREPQVYTLPPSREEMTKNQVSLTCLVKGFYPSDIAVEWESNGQPENNYKTTPPVLDSDGSFFLYSKLTVDKSRWQQGNVFSCSVMHEALHNHYTQKSLSLSPGK

SEQ ID NO: 103 - protein, 330 aa, synthetic construct
  REGION 1..330: note = Human IgG1 heavy chain constant region of IgG1G1m3 allotype
ASTKGPSVFPLAPSSKSTSGGTAALGCLVKDYFPEPVTVSWNSGALTSGVHTFPAVLQSSGLYSLSSVVTVPSSSLGTQTYICNVNHKPSNTKVDKRVEPKSCDKTHTCPPCPAPELLGGPSVFLFPPKPKDTLMISRTPEVTCVVVDVSHEDPEVKFNWYVDGVEVHNAKTKPREEQYNSTYRVVSVLTVLHQDWLNGKEYKCKVSNKALPAPIEKTISKAKGQPREPQVYTLPPSREEMTKNQVSLTCLVKGFYPSDIAVEWESNGQPENNYKTTPPVLDSDGSFFLYSKLTVDKSRWQQGNVFSCSVMHEALHNHYTQKSLSLSPGK

SEQ ID NO: 104 - protein, 107 aa, synthetic construct [sequence omitted]

SEQ ID NO: 105 - protein, 106 aa, synthetic construct
  REGION 1..106: note = Human kappa light chain constant region
TVAAPSVFIFPPSDEQLKSGTASVVCLLNNFYPREAKVQWKVDNALQSGNSQESVTEQDSKDSTYSLSSTLTLSKADYEKHKVYACEVTHQGLSSPVTKSFNRGEC

SEQ ID NO: 106 - DNA, 990 bp, synthetic construct
  misc_feature 1..990: note = Human IgG1 heavy chain constant region of IgG1G1m3 allotype
  source 1..990: mol_type = other DNA
gcctccaccaagggtccatcggtcttccccctggcaccctcctccaagagcacctctgggggcacagcggccctgggctgcctggtcaaggactacttccccgaaccggtgacggtgtcgtggaactcaggcgccctgaccagcggcgtgcacaccttcccggctgtcctacagtcctcaggactctactccctcagcagcgtggtgaccgtgccctccagcagcttgggcacccagacctacatctgcaacgtgaatcacaagcccagcaacaccaaggtggacaagagagttgagcccaaatcttgtgacaaaactcacacatgcccaccgtgcccagcacctgaactcctggggggaccgtcagtcttcctcttccccccaaaacccaaggacaccctcatgatctcccggacccctgaggtcacatgcgtggtggtggacgtgagccacgaagaccctgaggtcaagttcaactggtacgtggacggcgtggaggtgcataatgccaagacaaagccgcgggaggagcagtacaacagcacgtaccgtgtggtcagcgtcctcaccgtcctgcaccaggactggctgaatggcaaggagtacaagtgcaaggtctccaacaaagccctcccagcccccatcgagaaaaccatctccaaagccaaagggcagccccgagaaccacaggtgtacaccctgcccccatcccgggaggagatgaccaagaaccaggtcagcctgacctgcctggtcaaaggcttctatcccagcgacatcgccgtggagtgggagagcaatgggcagccggagaacaactacaagaccacgcctcccgtgctggactccgacggctccttcttcctctatagcaagctcaccgtggacaagagcaggtggcagcaggggaacgtcttctcatgctccgtgatgcatgaggctctgcacaaccactacacgcagaagagcctctccctgtccccgggtaaa

SEQ ID NO: 107 - DNA, 321 bp, synthetic construct
  misc_feature 1..321: note = Human kappa light chain constant region
  source 1..321: mol_type = other DNA
cgaactgtggctgcaccatctgtcttcatcttcccgccatctgatgagcagttgaaatctggaactgcctctgttgtgtgcctgctgaataacttctatcccagagaggccaaagtacagtggaaggtggataacgccctccaatcgggtaactcccaggagagtgtcacagagcaggacagcaaggacagcacctacagcctcagcagcaccctgacgctgagcaaagcagactacgagaaacacaaagtctacgcctgcgaagtcacccatcagggcctgagctcgcccgtcacaaagagcttcaacaggggagagtgt

SEQ ID NO: 108 - DNA, 318 bp, synthetic construct
  misc_feature 1..318: note = Human kappa light chain constant region
  source 1..318: mol_type = other DNA
actgtggctgcaccatctgtcttcatcttcccgccatctgatgagcagttgaaatctggaactgcctctgttgtgtgcctgctgaataacttctatcccagagaggccaaagtacagtggaaggtggataacgccctccaatcgggtaactcccaggagagtgtcacagagcaggacagcaaggacagcacctacagcctcagcagcaccctgacgctgagcaaagcagactacgagaaacacaaagtctacgcctgcgaagtcacccatcagggcctgagctcgcccgtcacaaagagcttcaacaggggagagtgt

SEQ ID NO: 109 - protein, 147 aa, Homo sapiens
MASHRLLLLCLAGLVFVSEAGPTGTGESKCPLMVKVLDAVRGSPAINVAVHVFRKAADDTWEPFASGKTSESGELHGLTTEEEFVEGIYKVEIDTKSYWKALGISPFHEHAEVVFTANDSGPRRYTIAALLSPYSYSTTAVVTNPKE

SEQ ID NO: 110 - protein, 127 aa, Homo sapiens
GPTGTGESKCPLMVKVLDAVRGSPAINVAVHVFRKAADDTWEPFASGKTSESGELHGLTTEEQFVEGIYKVEIDTKSYWKALGISPFHEHAEVVFTANDSGPRRYTIAALLSPYSYSTTAVVTNPKE

SEQ ID NO: 111 - protein, 127 aa, Homo sapiens; identical to SEQ ID NO: 110

SEQ ID NO: 112 - protein, 138 aa, Homo sapiens
MASHRLLLLCLAGLVFVSEAGPTGTGESKCPLMVKVLDAVRGSPAINVAVHVFRKAADDTWEPFASGKTSESGELHGLTTEEEFVEGIYKVEIDTKSYWKALGISPFHEHAEVVFTANDSGPRRYSYSTTAVVTNPKE

SEQ ID NO: 113 - protein, 9 aa, synthetic construct
  REGION 1..9: note = Transthyretin residues 89-97
EHAEVVFTA

SEQ ID NO: 114 - protein, 15 aa, synthetic construct
  REGION 1..15: note = Potential transthyretin immunogen
GGEHAEVVFTAGGKG

SEQ ID NO: 115 - protein, 12 aa, synthetic construct
  REGION 1..12: note = Potential transthyretin immunogen
CGGEHAEVVFTA

SEQ ID NO: 116 - protein, 12 aa, synthetic construct
  REGION 1..12: note = Potential transthyretin immunogen
EHAEVVFTACGG

SEQ ID NO: 117 - protein, 10 aa, synthetic construct
  REGION 1..10: note = 9D5 CDRH1 - Composite Chothia-Kabat
GFTFSSYTMS

SEQ ID NO: 118 - protein, 10 aa, synthetic construct
  REGION 1..10: note = 14G8 CDRH1 - Composite Chothia-Kabat
GFTFSSYTMS